European Patent Application EP 4 707 301 A1, published March 11, 2026. Title: IL-5RalphaXCD3epsilon T cell engaging bispecific antibody and Uses. Applicant: Ajou University Industry Academic Cooperation Foundation. The sequence listing filed with the application follows.

SEQUENCE LISTING (45 sequences)

SEQ ID NO: 1 - protein, 5 aa, synthetic construct
  REGION 1..5: note = Synthetic Sequence
SYWIN

SEQ ID NO: 2 - protein, 17 aa, synthetic construct
  REGION 1..17: note = Synthetic Sequence
HIYPNKNENYYNHKFKD

SEQ ID NO: 3 - protein, 13 aa, synthetic construct
  REGION 1..13: note = Synthetic Sequence
EFYGRQYYQAMDY

SEQ ID NO: 4 - protein, 11 aa, synthetic construct
  REGION 1..11: note = Synthetic Sequence
KASQNVGTAVA

SEQ ID NO: 5 - protein, 7 aa, synthetic construct
  REGION 1..7: note = Synthetic Sequence
WASTRHT

SEQ ID NO: 6 - protein, 9 aa, synthetic construct
  REGION 1..9: note = Synthetic Sequence
QQFGRYPYT

SEQ ID NO: 7 - protein, 5 aa, synthetic construct
  REGION 1..5: note = Synthetic Sequence
TYAMN

SEQ ID NO: 8 - protein, 19 aa, synthetic construct
  REGION 1..19: note = Synthetic Sequence
RIRSKYNNYATYYADSVKD

SEQ ID NO: 9 - protein, 14 aa, synthetic construct
  REGION 1..14: note = Synthetic Sequence
HGNFGNSYVSWFAY

SEQ ID NO: 10 - protein, 14 aa, synthetic construct
  REGION 1..14: note = Synthetic Sequence
RSSTGAVTTSNYAN

SEQ ID NO: 11 - protein, 7 aa, synthetic construct
  REGION 1..7: note = Synthetic Sequence
GTNKRAP

SEQ ID NO: 12 - protein, 9 aa, synthetic construct
  REGION 1..9: note = Synthetic Sequence
ALWYSNLWV

SEQ ID NO: 13 - protein, 5 aa, synthetic construct
  REGION 1..5: note = Synthetic Sequence
SYVIH

SEQ ID NO: 14 - protein, 17 aa, synthetic construct
  REGION 1..17: note = Synthetic Sequence
YINPYNDGTKYNERFKG

SEQ ID NO: 15 - protein, 12 aa, synthetic construct
  REGION 1..12: note = Synthetic Sequence
EGIRYYGLLGDY

SEQ ID NO: 16 - protein, 11 aa, synthetic construct
  REGION 1..11: note = Synthetic Sequence
GTSEDIINYLN

SEQ ID NO: 17 - protein, 7 aa, synthetic construct
  REGION 1..7: note = Synthetic Sequence
HTSRLQS

SEQ ID NO: 18 - protein, 9 aa, synthetic construct
  REGION 1..9: note = Synthetic Sequence
QQGYTLPYT

SEQ ID NO: 19 - protein, 13 aa, synthetic construct
  REGION 1..13: note = Synthetic Sequence
DYYGRSYYYAMDY

SEQ ID NO: 20 - protein, 122 aa, synthetic construct
  REGION 1..122: note = Synthetic Sequence
QVQLVQSGAEVKKPGSSVKVSCKASGYTFTSYWINWVRQAPGQGLEWIGHIYPNKNENYYNHKFKDKATLTVDKSTNTAYMELSSLRSEDTAVYYCTREFYGRQYYQAMDYWGQGTTLTVSS

SEQ ID NO: 21 - protein, 107 aa, synthetic construct
  REGION 1..107: note = Synthetic Sequence
DIQMTQSPSTLSASVGDRVTITCKASQNVGTAVAWYQQKPGKAPKLLIYWASTRHTGVPDRFSGSGSGTDFTLTISSLQPDDFATYYCQQFGRYPYTFGSGTKVEVK

SEQ ID NO: 22 - protein, 121 aa, synthetic construct [sequence omitted]

SEQ ID NO: 23 - protein, 107 aa, synthetic construct [sequence omitted]

SEQ ID NO: 24 - protein, 122 aa, synthetic construct
  REGION 1..122: note = Synthetic Sequence
QVQLVQSGAEVKKPGSSVKVSCKASGYTFTSYWINWVRQAPGQGLEWIGHIYPNKNENYYNHKFKDKATLTVDKSTNTAYMELSSLRSEDTAVYYCTRDYYGRSYYYAMDYWGQGTTLTVSS

SEQ ID NO: 25 - protein, 125 aa, synthetic construct
  REGION 1..125: note = Synthetic Sequence
EVQLVESGGGLVQPKGSLKLSCAASGFTFNTYAMNWVRQAPGKGLEWVARIRSKYNNYATYYADSVKDRFTISRDDSQSILYLQMNNLKTEDTAMYYCVRHGNFGNSYVSWFAYWGQGTLVTVSS

SEQ ID NO: 26 - protein, 109 aa, synthetic construct
  REGION 1..109: note = Synthetic Sequence
QAVVTQESALTTSPGETVTLTCRSSTGAVTTSNYANWVQEKPDHLFTGLIGGTNKRAPGVPARFSGSLIGDKAALTITGAQTEDEAIYFCALWYSNLWVFGGGTKLTVL

SEQ ID NO: 27 - protein, 482 aa, synthetic construct
  REGION 1..482: note = Synthetic Sequence
MGWSCIILFLVATATGVHSDIQMTQSPSTLSASVGDRVTITCKASQNVGTAVAWYQQKPGKAPKLLIYWASTRHTGVPDRFSGSGSGTDFTLTISSLQPDDFATYYCQQFGRYPYTFGSGTKVEVKGGGSGGGGEVQLVESGGGLVQPKGSLKLSCAASGFTFNTYAMNWVRQAPGKGLEWVARIRSKYNNYATYYADSVKDRFTISRDDSQSILYLQMNNLKTEDTAMYYCVRHGNFGNSYVSWFAYWGQGTLVTVSSGCPPCPAPEFEGGPSVFLFPPKPKDTLMISRTPEVTCVVVAVSHEDPEVKFNWYVDGVEVHNAKTKPREEQYNSTYRVVSVLTVLHQDWLNGKEYKCKVSNKALPAPIEKTISKAKGQPREPQVYTLPPSRDELTENQVSLTCLVKGFYPSDIAVEWESNGQPENNYKTTPPVLDSDGSFFLYSWLTVDKSRWQQGNVFSCSVMHEALHNHYTQKSLSLSPGK

SEQ ID NO: 28 - protein, 481 aa, synthetic construct
  REGION 1..481: note = Synthetic Sequence
MGWSCIILFLVATATGVHSQAVVTQESALTTSPGETVTLTCRSSTGAVTTSNYANWVQEKPDHLFTGLIGGTNKRAPGVPARFSGSLIGDKAALTITGAQTEDEAIYFCALWYSNLWVFGGGTKLTVLGGGSGGGGQVQLVQSGAEVKKPGSSVKVSCKASGYTFTSYWINWVRQAPGQGLEWIGHIYPNKNENYYNHKFKDKATLTVDKSTNTAYMELSSLRSEDTAVYYCTREFYGRQYYQAMDYWGQGTTLTVSSGCPPCPAPEFEGGPSVFLFPPKPKDTLMISRTPEVTCVVVAVSHEDPEVKFNWYVDGVEVHNAKTKPREEQYNSTYRVVSVLTVLHQDWLNGKEYKCKVSNKALPAPIEKTISKAKGQPREPRVYTLPPSRDELTKNQVSLTCLVKGFYPSDIAVEWESNGQPENNYKTTPPVLVSDGSFTLYSKLTVDKSRWQQGNVFSCSVMHEALHNHYTQKSLSLSPGK

SEQ ID NO: 29 - protein, 500 aa, synthetic construct
  REGION 1..500: note = Synthetic Sequence
MGWSCIILFLVATATGVHSQAVVTQESALTTSPGETVTLTCRSSTGAVTTSNYANWVQEKPDHLFTGLIGGTNKRAPGVPARFSGSLIGDKAALTITGAQTEDEAIYFCALWYSNLWVFGGGTKLTVLGGGGSGGGGSGGGGSEVQLVESGGGLVQPKGSLKLSCAASGFTFNTYAMNWVRQAPGKGLEWVARIRSKYNNYATYYADSVKDRFTISRDDSQSILYLQMNNLKTEDTAMYYCVRHGNFGNSYVSWFAYWGQGTLVTVSSEPKSCDKTHTCPPCPAPEFEGGPSVFLFPPKPKDTLMISRTPEVTCVVVAVSHEDPEVKFNWYVDGVEVHNAKTKPREEQYNSTYRVVSVLTVLHQDWLNGKEYKCKVSNKALPAPIEKTISKAKGQPREPQVYTLPPSRDELTENQVSLTCLVKGFYPSDIAVEWESNGQPENNYKTTPPVLDSDGSFFLYSWLTVDKSRWQQGNVFSCSVMHEALHNHYTQKSLSLSPGK

SEQ ID NO: 30 - protein, 495 aa, synthetic construct
  REGION 1..495: note = Synthetic Sequence
MGWSCIILFLVATATGVHSDIQMTQSPSTLSASVGDRVTITCKASQNVGTAVAWYQQKPGKAPKLLIYWASTRHTGVPDRFSGSGSGTDFTLTISSLQPDDFATYYCQQFGRYPYTFGSGTKVEVKGGGGSGGGGSGGGGSQVQLVQSGAEVKKPGSSVKVSCKASGYTFTSYWINWVRQAPGQGLEWIGHIYPNKNENYYNHKFKDKATLTVDKSTNTAYMELSSLRSEDTAVYYCTREFYGRQYYQAMDYWGQGTTLTVSSEPKSCDKTHTCPPCPAPEFEGGPSVFLFPPKPKDTLMISRTPEVTCVVVAVSHEDPEVKFNWYVDGVEVHNAKTKPREEQYNSTYRVVSVLTVLHQDWLNGKEYKCKVSNKALPAPIEKTISKAKGQPREPRVYTLPPSRDELTKNQVSLTCLVKGFYPSDIAVEWESNGQPENNYKTTPPVLVSDGSFTLYSKLTVDKSRWQQGNVFSCSVMHEALHNHYTQKSLSLSPGK

SEQ ID NO: 31 - protein, 495 aa, synthetic construct
  REGION 1..495: note = Synthetic Sequence
MGWSCIILFLVATATGVHSQVQLVQSGAEVKKPGSSVKVSCKASGYTFTSYWINWVRQAPGQGLEWIGHIYPNKNENYYNHKFKDKATLTVDKSTNTAYMELSSLRSEDTAVYYCTREFYGRQYYQAMDYWGQGTTLTVSSGGGGSGGGGSGGGGSDIQMTQSPSTLSASVGDRVTITCKASQNVGTAVAWYQQKPGKAPKLLIYWASTRHTGVPDRFSGSGSGTDFTLTISSLQPDDFATYYCQQFGRYPYTFGSGTKVEVKEPKSCDKTHTCPPCPAPEFEGGPSVFLFPPKPKDTLMISRTPEVTCVVVAVSHEDPEVKFNWYVDGVEVHNAKTKPREEQYNSTYRVVSVLTVLHQDWLNGKEYKCKVSNKALPAPIEKTISKAKGQPREPRVYTLPPSRDELTKNQVSLTCLVKGFYPSDIAVEWESNGQPENNYKTTPPVLVSDGSFTLYSKLTVDKSRWQQGNVFSCSVMHEALHNHYTQKSLSLSPGK

SEQ ID NO: 32 - protein, 749 aa, synthetic construct
  REGION 1..749: note = Synthetic Sequence
MGWSCIILFLVATATGVHSDIQMTQSPSTLSASVGDRVTITCKASQNVGTAVAWYQQKPGKAPKLLIYWASTRHTGVPDRFSGSGSGTDFTLTISSLQPDDFATYYCQQFGRYPYTFGSGTKVEVKGGGGSGGGGSGGGGSQVQLVQSGAEVKKPGSSVKVSCKASGYTFTSYWINWVRQAPGQGLEWIGHIYPNKNENYYNHKFKDKATLTVDKSTNTAYMELSSLRSEDTAVYYCTREFYGRQYYQAMDYWGQGTTLTVSSGGGGSEVQLVESGGGLVQPKGSLKLSCAASGFTFNTYAMNWVRQAPGKGLEWVARIRSKYNNYATYYADSVKDRFTISRDDSQSILYLQMNNLKTEDTAMYYCVRHGNFGNSYVSWFAYWGQGTLVTVSSGGGGSGGGGSGGGGSQAVVTQESALTTSPGETVTLTCRSSTGAVTTSNYANWVQEKPDHLFTGLIGGTNKRAPGVPARFSGSLIGDKAALTITGAQTEDEAIYFCALWYSNLWVFGGGTKLTVLEPKSCDKTHTCPPCPAPEFEGGPSVFLFPPKPKDTLMISRTPEVTCVVVAVSHEDPEVKFNWYVDGVEVHNAKTKPREEQYNSTYRVVSVLTVLHQDWLNGKEYKCKVSNKALPAPIEKTISKAKGQPREPQVYTLPPSRDELTENQVSLTCLVKGFYPSDIAVEWESNGQPENNYKTTPPVLDSDGSFFLYSWLTVDKSRWQQGNVFSCSVMHEALHNHYTQKSLSLSPGK

SEQ ID NO: 33 - protein, 251 aa, synthetic construct
  REGION 1..251: note = Synthetic Sequence
MGWSCIILFLVATATGVHSEPKSCDKTHTCPPCPAPEFEGGPSVFLFPPKPKDTLMISRTPEVTCVVVAVSHEDPEVKFNWYVDGVEVHNAKTKPREEQYNSTYRVVSVLTVLHQDWLNGKEYKCKVSNKALPAPIEKTISKAKGQPREPRVYTLPPSRDELTKNQVSLTCLVKGFYPSDIAVEWESNGQPENNYKTTPPVLVSDGSFTLYSKLTVDKSRWQQGNVFSCSVMHEALHNHYTQKSLSLSPGK

SEQ ID NO: 34 - protein, 471 aa, synthetic construct
  REGION 1..471: note = Synthetic Sequence
MGWSCIILFLVATATGVHSQVQLVQSGAEVKKPGSSVKVSCKASGYTFTSYWINWVRQAPGQGLEWIGHIYPNKNENYYNHKFKDKATLTVDKSTNTAYMELSSLRSEDTAVYYCTREFYGRQYYQAMDYWGQGTTLTVSSASTKGPSVFPLAPSSKSTSGGTAALGCLVKDYFPEPVTVSWNSGALTSGVHTFPAVLQSSGLYSLSSVVTVPSSSLGTQTYICNVNHKPSNTKVDKKVEPKSCDKTHTCPPCPAPEFEGGPSVFLFPPKPKDTLMISRTPEVTCVVVAVSHEDPEVKFNWYVDGVEVHNAKTKPREEQYNSTYRVVSVLTVLHQDWLNGKEYKCKVSNKALPAPIEKTISKAKGQPREPRVYTLPPSRDELTKNQVSLTCLVKGFYPSDIAVEWESNGQPENNYKTTPPVLVSDGSFTLYSKLTVDKSRWQQGNVFSCSVMHEALHNHYTQKSLSLSPGK

SEQ ID NO: 35 - protein, 233 aa, synthetic construct
  REGION 1..233: note = Synthetic Sequence
MGWSCIILFLVATATGVHSDIQMTQSPSTLSASVGDRVTITCKASQNVGTAVAWYQQKPGKAPKLLIYWASTRHTGVPDRFSGSGSGTDFTLTISSLQPDDFATYYCQQFGRYPYTFGSGTKVEVKRTVAAPSVFIFPPSDEQLKSGTASVKCLLNNFYPREAKVQWKVDNALQSGNSQESVTEQDSKDSTYSLSSTLTLSKADYEKHKVYACEVTHQGLSSPVTKSFNRGEC

SEQ ID NO: 36 - protein, 474 aa, synthetic construct
  REGION 1..474: note = Synthetic Sequence
MGWSCIILFLVATATGVHSEVQLVESGGGLVQPKGSLKLSCAASGFTFNTYAMNWVRQAPGKGLEWVARIRSKYNNYATYYADSVKDRFTISRDDSQSILYLQMNNLKTEDTAMYYCVRHGNFGNSYVSWFAYWGQGTLVTVSSASTKGPSVFPLAPSSKSTSGGTAALGCLVKDYFPEPVTVSWNSGALTSGVHTFPAVLQSSGLYSLKSVVTVPSSSLGTQTYICNVNHKPSNTKVDKKVEPKSCDKTHTCPPCPAPELLGGPSVFLFPPKPKDTLMISRTPEVTCVVVDVSHEDPEVKFNWYVDGVEVHNAKTKPREEQYNSTYRVVSVLTVLHQDWLNGKEYKCKVSNKALPAPIEKTISKAKGQPREPQVYTLPPSRDELTENQVSLTCLVKGFYPSDIAVEWESNGQPENNYKTTPPVLDSDGSFFLYSWLTVDKSRWQQGNVFSCSVMHEALHNHYTQKSLSLSPGK

SEQ ID NO: 37 - protein, 216 aa, synthetic construct
  REGION 1..216: note = Synthetic Sequence
QAVVTQESALTTSPGETVTLTCRSSTGAVTTSNYANWVQEKPDHLFTGLIGGTNKRAPGVPARFSGSLIGDKAALTITGAQTEDEAIYFCALWYSNLWVFGGGTKLTVLRTVAAPSVFIFPPSDEQLKSGTASVECLLNNFYPREAKVQWKVDNALQSGNSQESVTEQDSKDSTYSLSSTLTLSKADYEKHKVYACEVTHQGLSSPVTKSFNRGEC

SEQ ID NO: 38 - protein, 749 aa, synthetic construct
  REGION 1..749: note = Synthetic Sequence
MGWSCIILFLVATATGVHSDIQMTQSPSTLSASVGDRVTITCKASQNVGTAVAWYQQKPGKAPKLLIYWASTRHTGVPDRFSGSGSGTDFTLTISSLQPDDFATYYCQQFGRYPYTFGSGTKVEVKGGGGSGGGGSGGGGSQVQLVQSGAEVKKPGSSVKVSCKASGYTFTSYWINWVRQAPGQGLEWIGHIYPNKNENYYNHKFKDKATLTVDKSTNTAYMELSSLRSEDTAVYYCTREFYGRQYYQAMDYWGQGTTLTVSSGGGGSQAVVTQESALTTSPGETVTLTCRSSTGAVTTSNYANWVQEKPDHLFTGLIGGTNKRAPGVPARFSGSLIGDKAALTITGAQTEDEAIYFCALWYSNLWVFGGGTKLTVLGGGGSGGGGSGGGGSEVQLVESGGGLVQPKGSLKLSCAASGFTFNTYAMNWVRQAPGKGLEWVARIRSKYNNYATYYADSVKDRFTISRDDSQSILYLQMNNLKTEDTAMYYCVRHGNFGNSYVSWFAYWGQGTLVTVSSEPKSCDKTHTCPPCPAPEFEGGPSVFLFPPKPKDTLMISRTPEVTCVVVAVSHEDPEVKFNWYVDGVEVHNAKTKPREEQYNSTYRVVSVLTVLHQDWLNGKEYKCKVSNKALPAPIEKTISKAKGQPREPQVYTLPPSRDELTENQVSLTCLVKGFYPSDIAVEWESNGQPENNYKTTPPVLDSDGSFFLYSWLTVDKSRWQQGNVFSCSVMHEALHNHYTQKSLSLSPGK

SEQ ID NO: 39 - protein, 740 aa, synthetic construct
  REGION 1..740: note = Synthetic Sequence
MGWSCIILFLVATATGVHSDIQMTQSPSTLSASVGDRVTITCKASQNVGTAVAWYQQKPGKAPKLLIYWASTRHTGVPDRFSGSGSGTDFTLTISSLQPDDFATYYCQQFGRYPYTFGSGTKVEVKGGGGSGGGGSGGGGSQVQLVQSGAEVKKPGSSVKVSCKASGYTFTSYWINWVRQAPGQGLEWIGHIYPNKNENYYNHKFKDKATLTVDKSTNTAYMELSSLRSEDTAVYYCTREFYGRQYYQAMDYWGQGTTLTVSSGGGGSEVQLVESGGGLVQPKGSLKLSCAASGFTFNTYAMNWVRQAPGKGLEWVARIRSKYNNYATYYADSVKDRFTISRDDSQSILYLQMNNLKTEDTAMYYCVRHGNFGNSYVSWFAYWGQGTLVTVSSGGGGSGGGGSGGGGSQAVVTQESALTTSPGETVTLTCRSSTGAVTTSNYANWVQEKPDHLFTGLIGGTNKRAPGVPARFSGSLIGDKAALTITGAQTEDEAIYFCALWYSNLWVFGGGTKLTVLGCPPCPAPEFEGGPSVFLFPPKPKDTLMISRTPEVTCVVVAVSHEDPEVKFNWYVDGVEVHNAKTKPREEQYNSTYRVVSVLTVLHQDWLNGKEYKCKVSNKALPAPIEKTISKAKGQPREPQVYTLPPSRDELTENQVSLTCLVKGFYPSDIAVEWESNGQPENNYKTTPPVLDSDGSFFLYSWLTVDKSRWQQGNVFSCSVMHEALHNHYTQKSLSLSPGK

SEQ ID NO: 40 - protein, 486 aa, synthetic construct
  REGION 1..486: note = Synthetic Sequence
MGWSCIILFLVATATGVHSDIQMTQSPSTLSASVGDRVTITCKASQNVGTAVAWYQQKPGKAPKLLIYWASTRHTGVPDRFSGSGSGTDFTLTISSLQPDDFATYYCQQFGRYPYTFGSGTKVEVKGGGGSGGGGSGGGGSQVQLVQSGAEVKKPGSSVKVSCKASGYTFTSYWINWVRQAPGQGLEWIGHIYPNKNENYYNHKFKDKATLTVDKSTNTAYMELSSLRSEDTAVYYCTREFYGRQYYQAMDYWGQGTTLTVSSGCPPCPAPEFEGGPSVFLFPPKPKDTLMISRTPEVTCVVVAVSHEDPEVKFNWYVDGVEVHNAKTKPREEQYNSTYRVVSVLTVLHQDWLNGKEYKCKVSNKALPAPIEKTISKAKGQPREPRVYTLPPSRDELTKNQVSLTCLVKGFYPSDIAVEWESNGQPENNYKTTPPVLVSDGSFTLYSKLTVDKSRWQQGNVFSCSVMHEALHNHYTQKSLSLSPGK

SEQ ID NO: 41 - protein, 482 aa, synthetic construct
  REGION 1..482: note = Synthetic Sequence
MGWSCIILFLVATATGVHSDIQMTQSPSSLSASVGDRVTITCRASQDVNTAVAWYQQKPGKAPKLLIYSASFLYSGVPSRFSGSRSGTDFTLTISSLQPEDFATYYCQQHYTTPPTFGQGTKVEIKGGGSGGGGEVQLVESGGGLVQPKGSLKLSCAASGFTFNTYAMNWVRQAPGKGLEWVARIRSKYNNYATYYADSVKDRFTISRDDSQSILYLQMNNLKTEDTAMYYCVRHGNFGNSYVSWFAYWGQGTLVTVSSGCPPCPAPEFEGGPSVFLFPPKPKDTLMISRTPEVTCVVVAVSHEDPEVKFNWYVDGVEVHNAKTKPREEQYNSTYRVVSVLTVLHQDWLNGKEYKCKVSNKALPAPIEKTISKAKGQPREPQVYTLPPSRDELTENQVSLTCLVKGFYPSDIAVEWESNGQPENNYKTTPPVLDSDGSFFLYSWLTVDKSRWQQGNVFSCSVMHEALHNHYTQKSLSLSPGK

SEQ ID NO: 42 - protein, 214 aa, synthetic construct
  REGION 1..214: note = Synthetic Sequence
DIQMTQSPSSLSASVGDRVTITCRASQDVNTAVAWYQQKPGKAPKLLIYSASFLYSGVPSRFSGSRSGTDFTLTISSLQPEDFATYYCQQHYTTPPTFGQGTKVEIKRTVAAPSVFIFPPSDEQLKSGTASVKCLLNNFYPREAKVQWKVDNALQSGNSQESVTEQDSKDSTYSLSSTLTLSKADYEKHKVYACEVTHQGLSSPVTKSFNRGEC

SEQ ID NO: 43 - protein, 475 aa, synthetic construct
  REGION 1..475: note = Synthetic Sequence
DIQMTQSPSSLSASVGDRVTITCGTSEDIINYLNWYQQKPGKAPKLLIYHTSRLQSGVPSRFSGSGSGTDFTLTISSLQPEDFATYYCQQGYTLPYTFGQGTKVEIKGGGGSGGGGSGGGGSEVQLVQSGAEVKKPGASVKVSCKASGYTFTSYVIHWVRQRPGQGLAWMGYINPYNDGTKYNERFKGKVTITSDRSTSTVYMELSSLRSEDTAVYLCGREGIRYYGLLGDYWGQGTLVTVSSEPKSCDKTHTCPPCPAPEFEGGPSVFLFPPKPKDTLMISRTPEVTCVVVAVSHEDPEVKFNWYVDGVEVHNAKTKPREEQYNSTYRVVSVLTVLHQDWLNGKEYKCKVSNKALPAPIEKTISKAKGQPREPRVYTLPPSRDELTKNQVSLTCLVKGFYPSDIAVEWESNGQPENNYKTTPPVLVSDGSFTLYSKLTVDKSRWQQGNVFSCSVMHEALHNHYTQKSLSLSPGK

SEQ ID NO: 44 - protein, 476 aa, synthetic construct
  REGION 1..476: note = Synthetic Sequence
DIQMTQSPSTLSASVGDRVTITCKASQNVGTAVAWYQQKPGKAPKLLIYWASTRHTGVPDRFSGSGSGTDFTLTISSLQPDDFATYYCQQFGRYPYTFGSGTKVEVKGGGGSGGGGSGGGGSQVQLVQSGAEVKKPGSSVKVSCKASGYTFTSYWINWVRQAPGQGLEWIGHIYPNKNENYYNHKFKDKATLTVDKSTNTAYMELSSLRSEDTAVYYCTRDYYGRSYYYAMDYWGQGTTLTVSSEPKSCDKTHTCPPCPAPEFEGGPSVFLFPPKPKDTLMISRTPEVTCVVVAVSHEDPEVKFNWYVDGVEVHNAKTKPREEQYNSTYRVVSVLTVLHQDWLNGKEYKCKVSNKALPAPIEKTISKAKGQPREPRVYTLPPSRDELTKNQVSLTCLVKGFYPSDIAVEWESNGQPENNYKTTPPVLVSDGSFTLYSKLTVDKSRWQQGNVFSCSVMHEALHNHYTQKSLSLSPGK

SEQ ID NO: 45 - protein, 473 aa, synthetic construct
  REGION 1..473: note = Synthetic Sequence
DIQMTQSPSSLSASVGDRVTITCRASQDVNTAVAWYQQKPGKAPKLLIYSASFLYSGVPSRFSGSRSGTDFTLTISSLQPEDFATYYCQQHYTTPPTFGQGTKVEIKGGGGSGGGGSGGGGEVQLVESGGGLVQPGGSLRLSCAASGFNIKDTYIHWVRQAPGKGLEWVARIYPTNGYTRYADSVKGRFTISADTSKNTAYLQMNSLRAEDTAVYYCSRWGGDGFYAMDYWGQGTLVTVSSEPKSCDKTHTCPPCPAPEFEGGPSVFLFPPKPKDTLMISRTPEVTCVVVAVSHEDPEVKFNWYVDGVEVHNAKTKPREEQYNSTYRVVSVLTVLHQDWLNGKEYKCKVSNKALPAPIEKTISKAKGQPREPRVYTLPPSRDELTKNQVSLTCLVKGFYPSDIAVEWESNGQPENNYKTTPPVLVSDGSFTLYSKLTVDKSRWQQGNVFSCSVMHEALHNHYTQKSLSLSPGK